European Patent Application EP 4 755 889 A1, published June 10, 2026. Title: 아밀로이드-베타 올리고머 검출을 위한 화합물 및 이를 이용한 퇴행성 뇌질환을 진단하는 방법. Applicant: 아밀로이드솔루션 주식회사. Application KR. The sequence listing filed with the application follows.

SEQUENCE LISTING (3 sequences)

SEQ ID NO: 1 - protein, 7 aa, synthetic construct
FFAEDVG

SEQ ID NO: 2 - protein, 8 aa, synthetic construct
MVGGVVIA

SEQ ID NO: 3 - protein, 8 aa, synthetic construct
DAEFRHDS